European Patent Application EP 4 574 147 A1, published June 25, 2025. Title: 스테포게닌을 유효성분으로 포함하는 암 예방, 개선, 또는 치료용 조성물. Applicant: 경북대학교 산학협력단. The sequence listing filed with the application follows.

SEQUENCE LISTING (10 sequences)

SEQ ID NO: 1 - DNA, 18 bp, synthetic construct
  source 1..18: mol_type = other DNA
accatgaactttctgctc

SEQ ID NO: 2 - DNA, 18 bp, synthetic construct
  source 1..18: mol_type = other DNA
ggacggcttgaagatata

SEQ ID NO: 3 - DNA, 20 bp, synthetic construct
  source 1..20: mol_type = other DNA
attggctccggtatcgtcaa

SEQ ID NO: 4 - DNA, 20 bp, synthetic construct
  source 1..20: mol_type = other DNA
atggccacgatgctcagata

SEQ ID NO: 5 - DNA, 20 bp, synthetic construct
  source 1..20: mol_type = other DNA
ctgagaagcatgacggacaa

SEQ ID NO: 6 - DNA, 20 bp, synthetic construct
  source 1..20: mol_type = other DNA
cgccaacatagaccaccttt

SEQ ID NO: 7 - DNA, 20 bp, synthetic construct
  source 1..20: mol_type = other DNA
gtgtagtcagagacccctca

SEQ ID NO: 8 - DNA, 20 bp, synthetic construct
  source 1..20: mol_type = other DNA
ggaagaaaacagtgcctatg

SEQ ID NO: 9 - DNA, 18 bp, synthetic construct
  source 1..18: mol_type = other DNA
gactacctcatgaagatc

SEQ ID NO: 10 - DNA, 18 bp, synthetic construct
  source 1..18: mol_type = other DNA
gatccacatctgctggaa